European Patent Specification EP 3 541 832 B1, published July 22, 2026. Title: COMPOUNDS WITH ANTI-TUMOR ACTIVITY AGAINST CANCER CELLS BEARING EGFR OR HER2 EXON 20 MUTATIONS. Applicant: BOARD OF REGENTS, THE UNIVERSITY OF TEXAS SYSTEM Robichaux, Jacqulyne Nilsson, Monique Heymach, John  V. The sequence listing filed with the application follows.

SEQUENCE LISTING (18 sequences)

SEQ ID NO: 1 - protein, 4 aa, Artificial Sequence
  EGFR mutation
FQEA

SEQ ID NO: 2 - DNA, 12 bp, Artificial Sequence
  EGFR mutation
tccaggaagcct

SEQ ID NO: 3 - protein, 4 aa, Artificial Sequence
  HER2 mutation
YVMA

SEQ ID NO: 4 - DNA, 12 bp, Artificial Sequence
  HER2 mutation
tatgtcatggct

SEQ ID NO: 5 - DNA, 20 bp, Artificial Sequence
  Primer
cttacacccagtggagaagc

SEQ ID NO: 6 - DNA, 20 bp, Artificial Sequence
  Primer
accaagcgacggtcctccaa

SEQ ID NO: 7 - DNA, 45 bp, Homo sapiens
gaagcctacgtgatggccagcgtggacaacccccacgtgtgccgc

SEQ ID NO: 8 - DNA, 66 bp, Artificial Sequence
  EGFR exon 20 A763insFQEA
gaagcctccaggaagccttacgtgatggccagcagcgtggacgtggacaacccccacgtgtgccgc

SEQ ID NO: 9 - DNA, 45 bp, Artificial Sequence; identical to SEQ ID NO: 7
  EGFR exon 20 S768dupSVD

SEQ ID NO: 10 - DNA, 54 bp, Artificial Sequence
  EGFR exon 20 V769insASV
gaagcctacgtgatggccagcgtgccagcgtgggacaacccccacgtgtgccgc

SEQ ID NO: 11 - DNA, 54 bp, Artificial Sequence
  EGFR exon 20 D770insSVD
gaagcctacgtgatggccagcgtggacgcgtggacaaacccccacgtgtgccgc

SEQ ID NO: 12 - DNA, 54 bp, Artificial Sequence
  EGFR exon 20 H773insNPH
gaagcctacgtgatggccagcgtggacaacccccacaacccccacgtgtgccgc

SEQ ID NO: 13 - DNA, 48 bp, Homo sapiens
gaagcatacgtgatggctggtgtgggctccccatatgtctcccgcctt

SEQ ID NO: 14 - DNA, 48 bp, Artificial Sequence
  HER2 exon 20 G776V
gaagcatacgtgatggctgttgtgggctccccatatgtctcccgcctt

SEQ ID NO: 15 - DNA, 51 bp, Artificial Sequence
  HER2 exon 20 G776V V777insV
gaagcatacgtgatggcttgtgtgttgggctccccatatgtctcccgcctt

SEQ ID NO: 16 - DNA, 51 bp, Artificial Sequence
  HER2 exon 20 G776del insVV
gaagcatacgtgatggctgttgttgtgggctccccatatgtctcccgcctt

SEQ ID NO: 17 - DNA, 52 bp, Artificial Sequence
  HER2 exon 20 G776del ins V
cgaagcatacgtgatggctggtgtgtctggctccccatatgtctcccgcctt

SEQ ID NO: 18 - DNA, 57 bp, Artificial Sequence
  HER2 exon P780insGSP
gaagcatacgtgatggctggtgtgggctccccatggctcccctatgtctcccgcctt